European Patent Specification EP 3 307 753 B1, published January 24, 2024. Title: UV-B absorbing compounds isolated from plants. Applicant: MAX-PLANCK-GESELLSCHAFT zur FÖRDERUNG der WISSENSCHAFTEN e.V. The sequence listing filed with the application follows.

SEQUENCE LISTING (22 sequences)

SEQ ID NO: 1 - DNA, 1305 bp, Artificial Sequence
  cDNA of C24 FPT2
atgagaactttttcacccaagttgctgcttcttcttttacttgttttaagacatcatgctgaatctggctctatcgtcaagtttcttcccggttttgaaggccctcttcctttcgaacttgaaaccgggtacatcggtattggtgaagaagaagaactgcaatcgttttactatttcattaagtctgagaagaatccaaaagaagatcctcttcttctttggatatctggaggacctggttgctcttctatttctgctcttctttttgagaatggacctgtggctctaaagttcgaggtttacaatgaaactctcccttatttggtctctactacatattcatggaccaagatgacgaacgtattattcttggatcagcctattggagttggcttctcctacaaaagaactccaaatcttgataaatcgagtgacacaatagaagtattgcggatatacgaatttcttcagaagtggctaggtgaacatcctgagtttttctccaacactttttacgtaggaggagattcttattccggtaagattgttccagctatcgttgataaaatctcacaagaaaattatttgtgctgcaaacctccaataaatcttcagggttatgttctcggaaacccaataacaaatttggaatctgattctaactatcgtattccatatgctcatggaatggcattaatttctgatgagctctacgaatccctgaagagaaactgcaaaggaagatataaaaccgtggatccatctaacaaaaaatgtttgaaacttgttgaaaaatacaataagtgttctgataaaatatttagagaactaatattattaccacagtgtgatgaaagatctccactctgctggggctaccacagtacactagctaaatattgggccaatgacgagagggtacgtgaagctcttcaaataagaaagggaagtataggaaaatggatacgatgtaatacgaatatacattacggtgacgacattattagcagcataccatatcatatgaataacagcatcaacggataccgatctctcatttacagtggtgatcacgatatggaggtacctttccttgcaactgaagcttggataagatctctcaattatcctattattgatgattggaggccttggataataaacaatcagatttcaggatacacgatgacctatgccaataagatgacatatgctactatcaagggaggtggacacactgcagagtataaaccagcggagagctttatcatgttccaacgatggatcagtggccagtctctgtaa

SEQ ID NO: 2 - protein, 434 aa, Arabidopsis thaliana
  MISC_FEATURE (1)..(434): amino acid sequence coded by SEQ-ID No. 1
MRTFSPKLLLLLLLVLRHHAESGSIVKFLPGFEGPLPFELETGYIGIGEEEELQSFYYFIKSEKNPKEDPLLLWISGGPGCSSISALLFENGPVALKFEVYNETLPYLVSTTYSWTKMTNVLFLDQPIGVGFSYKRTPNLDKSSDTIEVLRIYEFLQKWLGEHPEFFSNTFYVGGDSYSGKIVPAIVDKISQENYLCCKPPINLQGYVLGNPITNLESDSNYRIPYAHGMALISDELYESLKRNCKGRYKTVDPSNKKCLKLVEKYNKCSDKIFRELILLPQCDERSPLCWGYHSTLAKYWANDERVREALQIRKGSIGKWIRCNTNIHYGDDIISSIPYHMNNSINGYRSLIYSGDHDMEVPFLATEAWIRSLNYPIIDDWRPWIINNQISGYTMTYANKMTYATIKGGGHTAEYKPAESFIMFQRWISGQSL

SEQ ID NO: 3 - DNA, 1227 bp, Artificial Sequence
  cDNA of C24 FPT1
atgaaatcaacactaaaattgctgcttctgcttctgtttatgttaaaccatcatgttgattctggctctatcgtcaagtttcttcccggctttgaaggccctcttcctttcgaactcgaaaccgggtacattggtattggtgaggaagaggaagtacagttgttctactactttataaagtctgagagaaatccaaaagaagaccctcttcttctctggttaagtggaggacctggatgttcatctatcactggccttcttttcgagaatggacctttggctttgaagtccgaggtttacaatggaagtgtcccttctttggtctctactacatattcgtggacaaagacggcgaacataatattcttggatcagcctattggagctggcttctcctactcaagaatcccacttattgatacgcctagtgacacaggcgaagttaagaatatccatgagtttctccaaaagtggttaagcaagcatccacagttttcttccaatcctttctatgctagcggagattcttattccggtatgattgttccagccctcgttcaagaaatttcgaaaggaaattatatatgttgcaaacctcctataaatctacagggctatatactcgggaacccaataacatattttgaagtcgaccaaaactatcgcattccattttctcatggaatggcacttatttcagatgaactatacgagtcaattaggagagactgcaaaggaaattatttcaacgtggatccacgtaacacaaaatgtttgaaacttgttgaagaataccataagtgtaccgacgaactaaatgaattcaatatattatcaccagattgcgacacgacatctcctgattgctttgtatatccatattatctccttggctactggatcaacgacgagagcgttcgcgatgctcttcatgttaataagagcagtattggaaaatgggagcgatgtacttatcaaaatagaatcccatacaacaaagacatcaataacagcataccataccatatgaataacagtattagtggctaccgatctctcatctacagtggtgatcatgatttggtggttcctttccttgcaactcaagcctggataaaatctctaaattactccatcattcatgaatggagaccttggatgattaaagatcaaatcgctgggtatataatatatttttgtgttatacacgagaacttattccaataa

SEQ ID NO: 4 - protein, 408 aa, Arabidopsis thaliana
  MISC_FEATURE (1)..(408): amino acid sequence coded by SEQ-ID No. 3
MKSTLKLLLLLLFMLNHHVDSGSIVKFLPGFEGPLPFELETGYIGIGEEEEVQLFYYFIKSERNPKEDPLLLWLSGGPGCSSITGLLFENGPLALKSEVYNGSVPSLVSTTYSWTKTANIIFLDQPIGAGFSYSRIPLIDTPSDTGEVKNIHEFLQKWLSKHPQFSSNPFYASGDSYSGMIVPALVQEISKGNYICCKPPINLQGYILGNPITYFEVDQNYRIPFSHGMALISDELYESIRRDCKGNYFNVDPRNTKCLKLVEEYHKCTDELNEFNILSPDCDTTSPDCFVYPYYLLGYWINDESVRDALHVNKSSIGKWERCTYQNRIPYNKDINNSIPYHMNNSISGYRSLIYSGDHDLVVPFLATQAWIKSLNYSIIHEWRPWMIKDQIAGYIIYFCVIHENLFQ

SEQ ID NO: 5 - DNA, 23 bp, Artificial Sequence
  forward primer for amplification of FPT2 cDNA (At2g22960)
atgagaactttttcacccaagtt

SEQ ID NO: 6 - DNA, 23 bp, Artificial Sequence
  reverse primer for amplification of FPT2 cDNA (At2g22960)
tcatcatctcttattattacaga

SEQ ID NO: 7 - DNA, 737 bp, Artificial Sequence
  cDNA of Col0 FPT2-1
atgagaactttttcacccaagttgctgcttcttcttttacttgttttaagacatcatgctgaatctggctctatcgtcaagtttcttcccggttttgaaggccctcttcctttcgaacttgaaaccggggctaccacagtacactagctaaatattgggccaatgacgagagggtacgtgaagctcttcaaataagaaagggaagtataggaaaatggatacgatgtaattcgaatatacattacgatgacgacattattagcagcataccatatcatatgaataacagcatcaacggataccgatctcttatttacaggtttgattaaaattacattttaaagaatcgatctagttctctatacaaactatgcggtttttggtaaacagtggtgatcacgatatggaggtacctttccttgcaactgaagcttggataagatctcttaattatcctattattgatgattggaggccttggataataaacaatcagattgctgggtgaataatttttacaatttttttttttgcttctttattcattaactcagtcgaatcatgagctcattagtcattttgaaatccctcttacgattttcttggacagatacacgatgacctatgccaataagatgacatatgctactatcaagggaggtggacacactgcagagtataaaccagcggagagctttatcatgttccaacgatggatcagtggccagcctctgtaa

SEQ ID NO: 8 - DNA, 651 bp, Artificial Sequence
  cDNA of Col0 FPT2-2
atgagaactttttcacccaagttgctgcttcttcttttacttgttttaagacatcatgctgaatctggctctatcgtcaagtttcttcccggttttgaaggccctcttcctttcgaacttgaaaccggggctaccacagtacactagctaaatattgggccaatgacgagagggtacgtgaagctcttcaaataagaaagggaagtataggaaaatggatacgatgtaattcgaatatacattacgatgacgacattattagcagcataccatatcatatgaataacagcatcaacggataccgatctcttatttacagtggtgatcacgatatggaggtacctttccttgcaactgaagcttggataagatctcttaattatcctattattgatgattggaggccttggataataaacaatcagattgctggatacacgatgacctatgccaataagatgacatatgctactatcaaggcaagttttttttttttgttcttactcttaatgttttttattacacaaatcattttgtttctcagtaactgttttgaggggtttactatagggaggtggacacactgcagagtataaaccagcggagagctttatcatgttccaacgatggatcagtggccagcctctgtaa

SEQ ID NO: 9 - DNA, 631 bp, Artificial Sequence
  cDNA of Col0 FPT2-3
atgagaactttttcacccaagttgctgcttcttcttttacttgttttaagacatcatgctgaatctggctctatcgtcaagtttcttcccggttttgaaggccctcttcctttcgaacttgaaaccggggctaccacagtacactagctaaatattgggccaatgacgagagggtacgtgaagctcttcaaataagaaagggaagtataggaaaatggatacgatgtaattcgaatatacattacgatgacgacattattagcagcataccatatcatatgaataacagcatcaacggataccgatctcttatttacaggtttgattaaaattacattttaaagaatcgatctagttctctatacaaactatgcggtttttggtaaacagtggtgatcacgatatggaggtacctttccttgcaactgaagcttggataagatctcttaattatcctattattgatgattggaggccttggataataaacaatcagattgctggatacacgatgacctatgccaataagatgacatatgctactatcaagggaggtggacacactgcagagtataaaccagcggagagctttatcatgttccaacgatggatcagtggccagcctctgtaa

SEQ ID NO: 10 - DNA, 560 bp, Artificial Sequence
  cDNA of Col0 FPT2-4
atgagaactttttcacccaagttgctgcttcttcttttacttgttttaagacatcatgctgaatctggctctatcgtcaagtttcttcccggttttgaaggccctcttcctttcgaacttgaaaccggggctaccacagtacactagctaaatattgggccaatgacgagagggtacgtgaagctcttcaaataagaaagggaagtataggaaaatggatacgatgtaattcgaatatacattacgatgacgacattattagcagcataccatatcatatgaataacagcatcaacggataccgatctcttatttacagtggtgatcacgatatggaggtacctttccttgcaactgaagcttggataagatctcttaattatcctattattgatgattggaggccttggataataaacaatcagattgctggatacacgatgacctatgccaataagatgacatatgctactatcaagggaggtggacacactgcagagtataaaccagcggagagctttatcatgttccaacgatggatcagtggccagcctctgtaa

SEQ ID NO: 11 - DNA, 24 bp, Artificial Sequence
  forward primer of set 1 for amplification of FPT2 genome sequence
tggactagtacgagaattgcaaag

SEQ ID NO: 12 - DNA, 20 bp, Artificial Sequence
  reverse primer of set 1 for amplification of FPT2 genome sequence
accgggaagaaacttgacga

SEQ ID NO: 13 - DNA, 18 bp, Artificial Sequence
  forward primer of set 2 for amplification of FPT2 genome sequence
cgtggagcgaccagtgat

SEQ ID NO: 14 - DNA, 20 bp, Artificial Sequence
  reverse primer of set 2 for amplification of FPT2 genome sequence
cttcacgtaccctctcgtca

SEQ ID NO: 15 - DNA, 21 bp, Artificial Sequence
  forward primer of set 3 for amplification of FPT2 genome sequence
cttatgcagggctaccacagt

SEQ ID NO: 16 - DNA, 22 bp, Artificial Sequence
  reverse primer of set 3 for amplification of FPT2 genome sequence
accactgtttaccaaaaaccgc

SEQ ID NO: 17 - DNA, 22 bp, Artificial Sequence
  forward primer of set 4 for amplification of FPT2 genome sequence
atatcatatgaataacagcatc

SEQ ID NO: 18 - DNA, 20 bp, Artificial Sequence
  reverse primer of set 4 for amplification of FPT2 genome sequence
gcatagggcatcatcatctc

SEQ ID NO: 19 - DNA, 19 bp, Artificial Sequence
  forward primer for amplification of FPT1 cDNA (At2g22920)
atgaaatcaacaccaaaat

SEQ ID NO: 20 - DNA, 23 bp, Artificial Sequence
  reverse primer for amplification of FPT1 cDNA (At2g22920)
atttaggtaaggtcattcaagta

SEQ ID NO: 21 - protein, 10 aa, Artificial Sequence
  amino acid (aa) sequence of a variant of BLOCK 1
  MISC_FEATURE (7)..(9): x = random amino acid
  MISC_FEATURE (7)..(9): Xaa can be any naturally occuring amino acid
GPGCSSXXXL

SEQ ID NO: 22 - protein, 6 aa, Arabidopsis thaliana
  MISC_FEATURE (1)..(6): amino acid (aa) sequence of a variant of BLOCK 2
GDSYSG